European Patent Application EP 4 541 821 A1, published April 23, 2025. Title: BISPECIFIC ANTIBODY CONTAINING ANTI-CLDN18.2 ANTIBODY, AND PHARMACEUTICAL COMPOSITION AND USE THEREOF. Applicant: AKESO BIOPHARMA, INC. Application WO PCT/CN2023/100452, filed June 15, 2023. The sequence listing filed with the application follows.

SEQUENCE LISTING (65 sequences)

SEQ ID NO: 1 - DNA, 351 bp, synthetic construct
  source 1..351: mol_type = other DNA; note = nucleic acid sequence encoding 6F7 heavy chain variable region
caggtgcagctgcagcagccaggagcagagctggtgaggccaggagcatccgtgaagctgtcttgtaaggccagcggctacaccttcacatcctattggatgaactgggtgaagcagaggcctggacagggactggagtggatcggcatgatcgacccaagcgattccgagacccacaacaatcagatgtttaaggacaaggccaccctgacagtggataagagctccaataccgcctacatgcacctgtctagcctgacatctgaggacagcgccgtgtatcactgcgcccggctgtacagatggtattttgacgtgtggggagcaggaaccacagtgaccgtgtcctct

SEQ ID NO: 2 - protein, 117 aa, synthetic construct
  source 1..117: note = 6F7 heavy chain variable region
QVQLQQPGAELVRPGASVKLSCKASGYTFTSYWMNWVKQRPGQGLEWIGMIDPSDSETHNNQMFKDKATLTVDKSSNTAYMHLSSLTSEDSAVYHCARLYRWYFDVWGAGTTVTVSS

SEQ ID NO: 3 - DNA, 321 bp, synthetic construct
  source 1..321: mol_type = other DNA; note = nucleic acid sequence encoding 6F7 light chain variable region
aacatcgtgatgacccagtcccccaagtctatgagcatgtccctgggcgagagggtgaccctgtcctgtaaggcctctgagatcgtgggcacatacgtgtcttggtttcagcagaagccacaccagagccccaagctgctgatctacggcgcctccaatcggtatacaggcgtgcctgacagattcaccggctctggcagcgccacagacttcaccctgacaatctctaacgtgcaggccgaggacctggccgattatcactgcggccagagctacaatttcccttatacctttggcggcggcacaaagctggagatcaag

SEQ ID NO: 4 - protein, 107 aa, synthetic construct
  source 1..107: note = 6F7 light chain variable region
NIVMTQSPKSMSMSLGERVTLSCKASEIVGTYVSWFQQKPHQSPKLLIYGASNRYTGVPDRFTGSGSATDFTLTISNVQAEDLADYHCGQSYNFPYTFGGGTKLEIK

SEQ ID NO: 5 - protein, 8 aa, synthetic construct
  source 1..8: note = 6F7CDR HCDR1
GYTFTSYW

SEQ ID NO: 6 - protein, 8 aa, synthetic construct
  source 1..8: note = 6F7CDR HCDR2
IDPSDSET

SEQ ID NO: 7 - protein, 10 aa, synthetic construct
  source 1..10: note = 6F7CDR HCDR3
ARLYRWYFDV

SEQ ID NO: 8 - protein, 6 aa, synthetic construct
  source 1..6: note = 6F7CDR LCDR1
EIVGTY

SEQ ID NO: 9 - skipped

SEQ ID NO: 10 - protein, 9 aa, synthetic construct
  source 1..9: note = 6F7CDR LCDR3
GQSYNFPYT

SEQ ID NO: 11 - DNA, 351 bp, synthetic construct
  source 1..351: mol_type = other DNA; note = nucleic acid sequence encoding 6F7H1VH
caggtgcagctggtgcagagcggagcagaggtggtgaagccaggagcctctgtgaagctgagctgtaaggcctccggctacaccttcacaagctattggatgaactgggtgcggcagagaccaggacagggactggagtggatcggaatgatcgacccttccgattctgagacccacaatgcccagaagtttcagggcaaggccaccctgacagtggacaagagcacctccacagcctacatgcacctgagctccctgcggtccgaggacacagccgtgtactattgcgccaggctgtaccgctggtattttgacgtgtggggagcaggaaccacagtgaccgtgtctagc

SEQ ID NO: 12 - protein, 117 aa, synthetic construct
  source 1..117: note = 6F7H1VH
QVQLVQSGAEVVKPGASVKLSCKASGYTFTSYWMNWVRQRPGQGLEWIGMIDPSDSETHNAQKFQGKATLTVDKSTSTAYMHLSSLRSEDTAVYYCARLYRWYFDVWGAGTTVTVSS

SEQ ID NO: 13 - DNA, 321 bp, synthetic construct
  source 1..321: mol_type = other DNA; note = nucleic acid sequence encoding 6F7L1VL
aacatcgtgatgacccagtccccagccacaatgtctatgagcccaggagagagggtgaccctgtcctgtagagcctctgagatcgtgggcacatacgtgtcttggtttcagcagaagccaggacaggcacctaggctgctgatctacggagcaagcaacaggtataccggagtgccagcacgcttctccggctctggcagcggcacagactttaccctgacaatcagctccgtgcagcctgaggacctggccgattatcactgcggccagtcttacaatttcccatatacctttggcggcggcacaaagctggagatcaag

SEQ ID NO: 14 - protein, 107 aa, synthetic construct
  source 1..107: note = 6F7L1VL
NIVMTQSPATMSMSPGERVTLSCRASEIVGTYVSWFQQKPGQAPRLLIYGASNRYTGVPARFSGSGSGTDFTLTISSVQPEDLADYHCGQSYNFPYTFGGGTKLEIK

SEQ ID NO: 15 - DNA, 351 bp, synthetic construct
  source 1..351: mol_type = other DNA; note = nucleic acid sequence encoding 6F7H2VH
caggtgcagctggtgcagagcggagcagaggtggtgaagccaggagcctctgtgaaggtgagctgtaaggcctccggctacaccttcacatcctattggatgaactgggtgcggcagagaccaggacagggactggagtggatcggaatcatcgacccttccgattctgagacctctaatgcccagaagtttcagggccgggtgaccctgacagtggacaagagcacctccacagcctacatgcacctgagctccctgaggagcgaggacacagccgtgtactattgcgccaggctgtaccgctggtattttgacgtgtggggagcaggaaccacagtgaccgtgtctagc

SEQ ID NO: 16 - protein, 117 aa, synthetic construct
  source 1..117: note = 6F7H2VH
QVQLVQSGAEVVKPGASVKVSCKASGYTFTSYWMNWVRQRPGQGLEWIGIIDPSDSETSNAQKFQGRVTLTVDKSTSTAYMHLSSLRSEDTAVYYCARLYRWYFDVWGAGTTVTVSS

SEQ ID NO: 17 - DNA, 321 bp, synthetic construct
  source 1..321: mol_type = other DNA; note = nucleic acid sequence encoding 6F7L2VL
aacatcgtgatgacccagtccccagccacactgtctctgagcccaggagagagggtgaccctgtcctgtagagcctctgagatcgtgggcacatacgtgtcttggtttcagcagaagccaggacaggcacctaggctgctgatctatggcgccagcaacagggcaaccggcatccccgcacgcttctccggctctggcagcggcacagactttaccctgacaatcagctccctgcagcctgaggacctggccgattactattgcggccagtcttacaatttcccatatacctttggcggcggcacaaagctggagatcaag

SEQ ID NO: 18 - protein, 107 aa, synthetic construct
  source 1..107: note = 6F7L2VL
NIVMTQSPATLSLSPGERVTLSCRASEIVGTYVSWFQQKPGQAPRLLIYGASNRATGIPARFSGSGSGTDFTLTISSLQPEDLADYYCGQSYNFPYTFGGGTKLEIK

SEQ ID NO: 19 - DNA, 351 bp, synthetic construct
  source 1..351: mol_type = other DNA; note = nucleic acid sequence encoding 6F7H3VH
caggtgcagctggtgcagagcggagcagaggtggtgaagccaggagcctctgtgaaggtgagctgtaaggcctccggctacaccttcacatcctattggatgaactgggtgcggcaggcaccaggacagggactggagtggatcggcatcatcgacccttccgattctgagacctcttacgcccagaagtttcagggcagggtgaccctgacagtggacaagagcacctccacagcctatatggagctgagctccctgcgcagcgaggacacagccgtgtactattgcgcccggctgtacagatggtattttgacgtgtggggagcaggaaccacagtgaccgtgtctagc

SEQ ID NO: 20 - protein, 117 aa, synthetic construct
  source 1..117: note = 6F7H3VH
QVQLVQSGAEVVKPGASVKVSCKASGYTFTSYWMNWVRQAPGQGLEWIGIIDPSDSETSYAQKFQGRVTLTVDKSTSTAYMELSSLRSEDTAVYYCARLYRWYFDVWGAGTTVTVSS

SEQ ID NO: 21 - DNA, 321 bp, synthetic construct
  source 1..321: mol_type = other DNA; note = nucleic acid sequence encoding 6F7L3VL
aacatcgtgatgacccagtccccagccacactgtctctgagcccaggagagagggtgaccctgtcctgtagagcctctgagatcgtgggcacatacctgtcttggtatcagcagaagccaggacaggcacctaggctgctgatctacggagccagcaccagggcaacaggcatccccgcacgcttctccggctctggcagcggcaccgactttaccctgacaatcagctccctgcagcctgaggattttgccgtgtactattgcggccagtcttacaatttcccatatacctttggcggcggcacaaagctggagatcaag

SEQ ID NO: 22 - protein, 107 aa, synthetic construct
  source 1..107: note = 6F7L3VL
NIVMTQSPATLSLSPGERVTLSCRASEIVGTYLSWYQQKPGQAPRLLIYGASTRATGIPARFSGSGSGTDFTLTISSLQPEDFAVYYCGQSYNFPYTFGGGTKLEIK

SEQ ID NO: 23 - DNA, 351 bp, synthetic construct
  source 1..351: mol_type = other DNA; note = nucleic acid sequence encoding 6F7H4VH
caggtgcagctggtgcagagcggagccgaagtggtgaagcctggcgcctctgtgaagctgtcctgtaaggcctctggctacacctttacatcctactggatgaactgggtgcggcagagaccaggccagtgcctggagtggatcggcatgatcgacccatctgattccgagacccacaatgcccagaagtttcagggcaaggccacactgaccgtggacaagagcacctccacagcctatatgcacctgtcctctctgagaagcgaggatacagccgtgtattactgtgccagactgtatcggtggtactttgacgtgtggggcgccggcaccacagtgaccgtgtctagc

SEQ ID NO: 24 - protein, 117 aa, synthetic construct
  source 1..117: note = 6F7H4VH
QVQLVQSGAEVVKPGASVKLSCKASGYTFTSYWMNWVRQRPGQCLEWIGMIDPSDSETHNAQKFQGKATLTVDKSTSTAYMHLSSLRSEDTAVYYCARLYRWYFDVWGAGTTVTVSS

SEQ ID NO: 25 - DNA, 321 bp, synthetic construct
  source 1..321: mol_type = other DNA; note = nucleic acid sequence encoding 6F7L4VL
aatatcgtgatgacccagtctcctgccacaatgtctatgagccctggcgagagagtgaccctgtcttgtagggccagcgagatcgtgggcacctacgtgagctggttccagcagaagccaggccaggccccaagactgctgatctatggcgccagcaaccggtatacaggcgtgcctgccagattttctggctccggctctggcaccgatttcacactgaccatctctagcgtgcagcccgaggatctggccgattaccactgtggccagtcctacaacttcccctatacattcgggtgcggcactaaactcgagatcaaa

SEQ ID NO: 26 - protein, 107 aa, synthetic construct
  source 1..107: note = 6F7L4VL
NIVMTQSPATMSMSPGERVTLSCRASEIVGTYVSWFQQKPGQAPRLLIYGASNRYTGVPARFSGSGSGTDFTLTISSVQPEDLADYHCGQSYNFPYTFGCGTKLEIK

SEQ ID NO: 27 - DNA, 354 bp, synthetic construct
  source 1..354: mol_type = other DNA; note = nucleic acid sequence encoding 8C5.1VH
gaagtgcagctggttgagagcggcggaggactggtgaaacctggaggatctctgaagctgagctgcgctgcttccggattcacttttagcaactccgccgtgagctgggtgagacaaacacctgagaagaggctggagtgggtggctacaatcacaagcggcgtgagctacacctactacctggactccgtgaggggcagattcacaatcagcagggacaacgccaagaacaccctgtacctgcagatgagcagcctgaggagcgaggataccgctatgtactactgtaccaggcagttcaagggcaacgccctggattactggggccaaggaacctctgtgacagtgagctcc

SEQ ID NO: 28 - protein, 118 aa, synthetic construct
  source 1..118: note = 8C5.1VH
EVQLVESGGGLVKPGGSLKLSCAASGFTFSNSAVSWVRQTPEKRLEWVATITSGVSYTYYLDSVRGRFTISRDNAKNTLYLQMSSLRSEDTAMYYCTRQFKGNALDYWGQGTSVTVSS

SEQ ID NO: 29 - DNA, 339 bp, synthetic construct
  source 1..339: mol_type = other DNA; note = nucleic acid sequence encoding 8C5.1VL
gacattgtgatgacccagtccccttcctccctgacagtgacagctggagagaaggtgacaatgtcctgcaagagcagccagagcctgctgaactccggaaatcagaagaactacctgacctggtaccagcagaagcccggacaaccacctaagctgctgatctactgggcctccaccagggaaagcggagttcctgatagattcaccggcagcggctccggaacagatttcacactgacaatcaacaacttccaggctgaggacctggccgtgtactactgtcagaacgactacttctaccctctgaccttcggcgccggaacaaagctggaactgaag

SEQ ID NO: 30 - protein, 113 aa, synthetic construct
  source 1..113: note = 8C5.1VL
DIVMTQSPSSLTVTAGEKVTMSCKSSQSLLNSGNQKNYLTWYQQKPGQPPKLLIYWASTRESGVPDRFTGSGSGTDFTLTINNFQAEDLAVYYCQNDYFYPLTFGAGTKLELK

SEQ ID NO: 31 - protein, 8 aa, synthetic construct
  source 1..8: note = 8C5.1 HCDR1
GFTFSNSA

SEQ ID NO: 32 - protein, 8 aa, synthetic construct
  source 1..8: note = 8C5.1 HCDR2
ITSGVSYT

SEQ ID NO: 33 - protein, 11 aa, synthetic construct
  source 1..11: note = 8C5.1 HCDR3
TRQFKGNALDY

SEQ ID NO: 34 - protein, 12 aa, synthetic construct
  source 1..12: note = 8C5.1 LCDR1
QSLLNSGNQKNY

SEQ ID NO: 35 - skipped

SEQ ID NO: 36 - protein, 9 aa, synthetic construct
  source 1..9: note = 8C5.1 LCDR3
QNDYFYPLT

SEQ ID NO: 37 - protein, 118 aa, synthetic construct
  source 1..118: note = 8C5.1 H1VH
EVQLVESGGGLVKPGGSLRLSCAASGFTFSNSAVSWVRQAPGKRLEWVATITSGVSYTYYLDSVRGRFTISRDNAKNSLYLQMNSLRAEDTAVYYCTRQFKGNALDYWGQGTSVTVSS

SEQ ID NO: 38 - DNA, 354 bp, synthetic construct
  source 1..354: mol_type = other DNA; note = nucleic acid sequence encoding 8C5.1 H1VH
gaggtgcagctggtggagagcggcggcggcctggtgaagcccggcggcagcctgaggctgtcctgcgccgcctctggcttcaccttttctaacagcgccgtgtcttgggtgaggcaggcacctggcaagcgcctggagtgggtggccaccatcacatccggcgtgtcttacacctactatctggacagcgtgcggggcagattcacaatcagcagagataacgccaagaacagcctgtatctgcagatgaactctctgcgggccgaggacaccgccgtgtactattgtacaagacagtttaagggcaatgccctggattactggggccagggcaccagcgtgacagtgagctcc

SEQ ID NO: 39 - protein, 118 aa, synthetic construct
  source 1..118: note = 8C5.1 H2VH
EVQLVESGGGLVKPGGSLRLSCAASGFTFSNSAVSWVRQAPGKGLEWVSTITSGVSYTYYADSVKGRFTISRDNAKNSLYLQMNSLRAEDTAVYYCTRQFKGNALDYWGQGTSVTVSS

SEQ ID NO: 40 - DNA, 354 bp, synthetic construct
  source 1..354: mol_type = other DNA; note = nucleic acid sequence encoding 8C5.1 H2VH
gaggtgcagctggtggagagcggcggcggcctggtgaagcccggcggcagcctgaggctgtcctgcgcagcatctggcttcaccttttctaacagcgccgtgtcttgggtgaggcaggcacctggcaagggactggagtgggtgagcaccatcacatccggcgtgtcttacacctactatgccgactccgtgaagggccggttcacaatcagcagagataacgccaagaacagcctgtatctgcagatgaactctctgagggccgaggacaccgccgtgtactattgtacacgccagtttaagggcaatgccctggattactggggccagggcaccagcgtgacagtgagctcc

SEQ ID NO: 41 - protein, 118 aa, synthetic construct
  source 1..118: note = 8C5.1 H3VH
EVQLVESGGGLVKPGGSLRLSCAASGFTFSNSAVSWVRQAPGKGLEWVSSITSGVSYTYYADSVKGRFTISRDNAKNSLYLQMNSLRAEDTAVYYCTRQFKGNALDYWGQGTSVTVSS

SEQ ID NO: 42 - DNA, 354 bp, synthetic construct
  source 1..354: mol_type = other DNA; note = nucleic acid sequence encoding 8C5.1 H3VH
gaggtgcagctggtggagagcggcggcggcctggtgaagcccggcggcagcctgaggctgtcctgcgcagcatctggcttcaccttttctaacagcgccgtgtcttgggtgaggcaggcacctggcaagggactggagtgggtgagctccatcacatccggcgtgtcttacacctactatgccgactccgtgaagggccggttcacaatcagcagagataacgccaagaacagcctgtatctgcagatgaactctctgagggccgaggacaccgccgtgtactattgtacacgccagtttaagggcaatgccctggattactggggccagggcaccagcgtgacagtgagctcc

SEQ ID NO: 43 - protein, 113 aa, synthetic construct
  source 1..113: note = 8C5.1 L1VL
DIVMTQSPSSLSVSPGERVTMSCKSSQSLLNSGNQKNYLTWYQQKPGQPPKLLIYWASTRESGVPDRFSGSGSGTDFTLTINSFQAEDVAVYYCQNDYFYPLTFGAGTKLELK

SEQ ID NO: 44 - DNA, 339 bp, synthetic construct
  source 1..339: mol_type = other DNA; note = nucleic acid sequence encoding 8C5.1 L1VL
gatatcgtgatgacccagagcccatctagcctgtccgtgtctccaggcgagagagtgaccatgagctgcaagtcttcccagagcctgctgaatagcggcaaccagaagaactacctgacatggtaccagcagaagccaggccagcctccaaagctgctgatctactgggccagcacaagagagagcggcgtgccagacagattctctggcagcggctctggcaccgacttcacactgaccatcaactccttccaggccgaggatgtggccgtgtattactgccagaacgattacttctatcccctgacattcggcgccggcacaaagctggagctgaag

SEQ ID NO: 45 - protein, 113 aa, synthetic construct
  source 1..113: note = 8C5.1 L2VL
DIVMTQSPSSLSVSPGERVTISCKSSQSLLNSGNQKNYLTWYQQKPGQPPKLLIYWASTRESGVPDRFSGSGSGTDFTLTISSFQAEDVAVYYCQNDYFYPLTFGAGTKLELK

SEQ ID NO: 46 - DNA, 339 bp, synthetic construct
  source 1..339: mol_type = other DNA; note = nucleic acid sequence encoding 8C5.1 L2VL
gacatcgtgatgacccagtctccaagctccctgagcgtgtccccaggagagagggtgacaatctcctgcaagtctagccagtctctgctgaacagcggcaatcagaagaactacctgacctggtatcagcagaagcctggccagccccctaagctgctgatctactgggcctccaccagggagtctggagtgccagacagattttctggcagcggctccggcacagatttcaccctgacaatctcctcttttcaggccgaggacgtggccgtgtactattgtcagaatgattacttctatcccctgacctttggcgccggcacaaagctggagctgaag

SEQ ID NO: 47 - protein, 113 aa, synthetic construct
  source 1..113: note = 8C5.1 L3VL
DIVMTQSPSSLSVSPGERVTISCKSSQSLLNSGNQKNYLAWYQQKPGQPPKLLIYWASTRESGVPDRFSGSGSGTDFTLTISSLQAEDVAVYYCQNDYFYPLTFGAGTKLELK

SEQ ID NO: 48 - DNA, 339 bp, synthetic construct
  source 1..339: mol_type = other DNA; note = nucleic acid sequence encoding 8C5.1 L3VL
gacatcgtgatgacccagtctccaagctccctgagcgtgtccccaggagagagggtgacaatctcctgcaagtctagccagtctctgctgaacagcggcaatcagaagaactacctggcctggtatcagcagaagcctggccagccccctaagctgctgatctactgggcctccaccagggagtctggagtgccagacagattctctggcagcggctccggcacagacttcaccctgacaatctcctctctgcaggccgaggacgtggccgtgtactattgtcagaatgattacttctatcccctgacctttggcgccggcacaaagctggagctgaag

SEQ ID NO: 49 - protein, 7 aa, synthetic construct
  source 1..7: note = Amino acid sequence of TEV
ENLYFQG

SEQ ID NO: 50 - protein, 20 aa, synthetic construct
  source 1..20: note = Amino acid sequence of Linker
GGGGSGGGGSGGGGSGGGGS

SEQ ID NO: 51 - protein, 244 aa, synthetic construct
  source 1..244: note = scFv sequence
QVQLVQSGAEVVKPGASVKLSCKASGYTFTSYWMNWVRQRPGQCLEWIGMIDPSDSETHNAQKFQGKATLTVDKSTSTAYMHLSSLRSEDTAVYYCARLYRWYFDVWGAGTTVTVSSGGGGSGGGGSGGGGSGGGGSNIVMTQSPATMSMSPGERVTLSCRASEIVGTYVSWFQQKPGQAPRLLIYGASNRYTGVPARFSGSGSGTDFTLTISSVQPEDLADYHCGQSYNFPYTFGCGTKLEIK

SEQ ID NO: 52 - protein, 232 aa, synthetic construct
  source 1..232: note = Hinge region-CH2 domain-CH3 domain comprising Knob mutation sites S354C and T366W
EPKSSDKTHTCPPCPAPELLGGPSVFLFPPKPKDTLMISRTPEVTCVVVDVSHEDPEVKFNWYVDGVEVHNAKTKPREEQYNSTYRVVSVLTVLHQDWLNGKEYKCKVSNKALPAPIEKTISKAKGQPREPQVYTLPPCRDELTKNQVSLWCLVKGFYPSDIAVEWESNGQPENNYKTTPPVLDSDGSFFLYSKLTVDKSRWQQGNVFSCSVMHEALHNHYTQKSLSLSPGK

SEQ ID NO: 53 - protein, 476 aa, synthetic construct
  source 1..476: note = full-length amino acid sequence of HC1
QVQLVQSGAEVVKPGASVKLSCKASGYTFTSYWMNWVRQRPGQCLEWIGMIDPSDSETHNAQKFQGKATLTVDKSTSTAYMHLSSLRSEDTAVYYCARLYRWYFDVWGAGTTVTVSSGGGGSGGGGSGGGGSGGGGSNIVMTQSPATMSMSPGERVTLSCRASEIVGTYVSWFQQKPGQAPRLLIYGASNRYTGVPARFSGSGSGTDFTLTISSVQPEDLADYHCGQSYNFPYTFGCGTKLEIKEPKSSDKTHTCPPCPAPELLGGPSVFLFPPKPKDTLMISRTPEVTCVVVDVSHEDPEVKFNWYVDGVEVHNAKTKPREEQYNSTYRVVSVLTVLHQDWLNGKEYKCKVSNKALPAPIEKTISKAKGQPREPQVYTLPPCRDELTKNQVSLWCLVKGFYPSDIAVEWESNGQPENNYKTTPPVLDSDGSFFLYSKLTVDKSRWQQGNVFSCSVMHEALHNHYTQKSLSLSPGK

SEQ ID NO: 54 - DNA, 1428 bp, synthetic construct
  source 1..1428: mol_type = other DNA; note = nucleic acid sequence encoding full-length HC1
caggtgcagctggtgcagagcggagccgaagtggtgaagcctggcgcctctgtgaagctgtcctgtaaggcctctggctacacctttacatcctactggatgaactgggtgcggcagagaccaggccagtgcctggagtggatcggcatgatcgacccatctgattccgagacccacaatgcccagaagtttcagggcaaggccacactgaccgtggacaagagcacctccacagcctatatgcacctgtcctctctgagaagcgaggatacagccgtgtattactgtgccagactgtatcggtggtactttgacgtgtggggcgccggcaccacagtgaccgtgtctagcggaggcggaggatctggaggaggaggcagtggcggagggggaagcggcggaggaggatcaaatatcgtgatgacccagtctcctgccacaatgtctatgagccctggcgagagagtgaccctgtcttgtagggccagcgagatcgtgggcacctacgtgagctggttccagcagaagccaggccaggccccaagactgctgatctatggcgccagcaaccggtatacaggcgtgcctgccagattttctggctccggctctggcaccgatttcacactgaccatctctagcgtgcagcccgaggatctggccgattaccactgtggccagtcctacaacttcccctatacattcgggtgcggcactaaactcgagatcaaagagcccaaatcctccgacaagacacacacctgtcccccctgtcctgctcccgaactcctcggagggccctccgtgtttctgttccctccaaagcctaaagatactctgatgattagtaggactcccgaagtcacctgtgtggtcgtggacgtgtcacacgaagatcctgaggtcaaattcaactggtacgtggacggcgtcgaggtgcataatgccaagaccaagccccgcgaggaacagtacaacagcacctatcgagtcgtgtccgtcctgacagtgctgcaccaggattggctgaacgggaaggagtataagtgcaaagtgagcaataaggctctgcccgcacctatcgagaagaccatttccaaggctaaaggacagccccgcgagcctcaggtgtacacactgcccccttgccgggacgaactgaccaagaaccaggtctccctgtggtgtctggtgaagggcttctacccaagcgatatcgccgtggagtgggaatccaatggacagcccgagaacaattacaagaccacaccacccgtgctggactccgatggcagcttcttcctgtattccaagctgacagtggacaagagccggtggcagcaggggaacgtcttcagttgctcagtgatgcacgaggccctgcacaatcattacactcagaagagcctgtccctgtctccaggcaaa

SEQ ID NO: 55 - protein, 329 aa, synthetic construct
  source 1..329: note = Constant region sequence comprising Hole mutation sites Y349C, T366S, L368A, and Y407V
ASTKGPSVFPLAPSSKSTSGGTAALGCLVKDYFPEPVTVSWNSGALTSGVHTFPAVLQSSGLYSLSSVVTVPSSSLGTQTYICNVNHKPSNTKVDKKVEPKSCDKTHTCPPCPAPELLGGPSVFLFPPKPKDTLMISRTPEVTCVVVDVSHEDPEVKFNWYVDGVEVHNAKTKPREEQYNSTYRVVSVLTVLHQDWLNGKEYKCKVSNKALPAPIEKTISKAKGQPREPQVCTLPPSRDELTKNQVSLSCAVKGFYPSDIAVEWESNGQPENNYKTTPPVLDSDGSFFLVSKLTVDKSRWQQGNVFSCSVMHEALHNHYTQKSLSLSPG

SEQ ID NO: 56 - protein, 447 aa, synthetic construct
  source 1..447: note = full-length amino acid sequence of HC2
EVQLVESGGGLVKPGGSLRLSCAASGFTFSNSAVSWVRQAPGKGLEWVSSITSGVSYTYYADSVKGRFTISRDNAKNSLYLQMNSLRAEDTAVYYCTRQFKGNALDYWGQGTSVTVSSASTKGPSVFPLAPSSKSTSGGTAALGCLVKDYFPEPVTVSWNSGALTSGVHTFPAVLQSSGLYSLSSVVTVPSSSLGTQTYICNVNHKPSNTKVDKKVEPKSCDKTHTCPPCPAPELLGGPSVFLFPPKPKDTLMISRTPEVTCVVVDVSHEDPEVKFNWYVDGVEVHNAKTKPREEQYNSTYRVVSVLTVLHQDWLNGKEYKCKVSNKALPAPIEKTISKAKGQPREPQVCTLPPSRDELTKNQVSLSCAVKGFYPSDIAVEWESNGQPENNYKTTPPVLDSDGSFFLVSKLTVDKSRWQQGNVFSCSVMHEALHNHYTQKSLSLSPG

SEQ ID NO: 57 - DNA, 1341 bp, synthetic construct
  source 1..1341: mol_type = other DNA; note = nucleic acid sequence encoding full-length of HC2
gaggtgcagctggtggagagcggcggcggcctggtgaagcccggcggcagcctgaggctgtcctgcgcagcatctggcttcaccttttctaacagcgccgtgtcttgggtgaggcaggcacctggcaagggactggagtgggtgagctccatcacatccggcgtgtcttacacctactatgccgactccgtgaagggccggttcacaatcagcagagataacgccaagaacagcctgtatctgcagatgaactctctgagggccgaggacaccgccgtgtactattgtacacgccagtttaagggcaatgccctggattactggggccagggcaccagcgtgacagtgagctccgcctccacaaaggggcccagcgtgtttcctctcgccccctcctccaaaagcaccagcggaggaaccgctgctctcggatgtctggtgaaggactacttccctgaacccgtcaccgtgagctggaatagcggcgctctgacaagcggagtccatacattccctgctgtgctgcaaagcagcggactctattccctgtccagcgtcgtcacagtgcccagcagcagcctgggcacccagacctacatctgtaacgtcaaccacaagccctccaacaccaaggtggacaagaaagtggagcccaaatcctgcgacaagacccatacctgcccaccttgtccagctccagagctgctgggaggaccaagcgtgttcctgtttccacccaagcctaaagacaccctgatgatcagcagaaccccagaggtcacatgtgtggtcgtggacgtgtcccacgaggaccccgaagtcaagtttaactggtacgtggatggcgtggaggtccataatgccaagaccaagccccgcgaagagcagtacaactcaacttatcgagtcgtgagcgtgctgaccgtcctgcaccaggactggctgaacggaaaggagtataagtgcaaagtgtctaacaaggccctgcctgctccaatcgagaagaccattagcaaggccaaaggccagcccagagaacctcaggtgtgcaccctgcctccaagcagggatgagctgacaaagaaccaggtcagcctgtcctgtgctgtgaaaggattctacccctccgacatcgcagtggagtgggaatctaatggccagcctgagaacaattataagaccacaccccctgtgctggattcagacggcagcttcttcctggtgagcaagctgactgtggataagtcaaggtggcagcagggcaacgtgttcagctgtagtgtgatgcacgaggccctgcacaatcattacacccagaaatcactgagcctgtcccccggg

SEQ ID NO: 58 - protein, 107 aa, synthetic construct [sequence omitted]

SEQ ID NO: 59 - protein, 220 aa, synthetic construct
  source 1..220: note = full-length amino acid sequence of L3
DIVMTQSPSSLSVSPGERVTISCKSSQSLLNSGNQKNYLAWYQQKPGQPPKLLIYWASTRESGVPDRFSGSGSGTDFTLTISSLQAEDVAVYYCQNDYFYPLTFGAGTKLELKRTVAAPSVFIFPPSDEQLKSGTASVVCLLNNFYPREAKVQWKVDNALQSGNSQESVTEQDSKDSTYSLSSTLTLSKADYEKHKVYACEVTHQGLSSPVTKSFNRGEC

SEQ ID NO: 60 - DNA, 660 bp, synthetic construct
  source 1..660: mol_type = other DNA; note = nucleic acid sequence encoding full-length amino acid sequence of L3
gacatcgtgatgacccagtctccaagctccctgagcgtgtccccaggagagagggtgacaatctcctgcaagtctagccagtctctgctgaacagcggcaatcagaagaactacctggcctggtatcagcagaagcctggccagccccctaagctgctgatctactgggcctccaccagggagtctggagtgccagacagattctctggcagcggctccggcacagacttcaccctgacaatctcctctctgcaggccgaggacgtggccgtgtactattgtcagaatgattacttctatcccctgacctttggcgccggcacaaagctggagctgaagcgtacggtggcagccccatctgtcttcatttttccccctagtgacgagcagctgaaatccggaacagcctctgtggtctgtctgctgaacaatttctaccctcgcgaagccaaggtgcagtggaaagtcgataacgctctgcagagtggcaattcacaggagagcgtgactgaacaggactccaaggattctacctatagtctgagctccactctgaccctgtccaaagcagattacgaaaagcacaaagtgtatgcctgtgaggtcacccaccaggggctgagttctccagtcaccaaatccttcaacagaggcgaatgt

SEQ ID NO: 61 - protein, 330 aa, synthetic construct
  source 1..330: note = Amino acid sequence of the heavy chain constant region of human hG1WT
ASTKGPSVFPLAPSSKSTSGGTAALGCLVKDYFPEPVTVSWNSGALTSGVHTFPAVLQSSGLYSLSSVVTVPSSSLGTQTYICNVNHKPSNTKVDKKVEPKSCDKTHTCPPCPAPELLGGPSVFLFPPKPKDTLMISRTPEVTCVVVDVSHEDPEVKFNWYVDGVEVHNAKTKPREEQYNSTYRVVSVLTVLHQDWLNGKEYKCKVSNKALPAPIEKTISKAKGQPREPQVYTLPPSREEMTKNQVSLTCLVKGFYPSDIAVEWESNGQPENNYKTTPPVLDSDGSFFLYSKLTVDKSRWQQGNVFSCSVMHEALHNHYTQKSLSLSPGK

SEQ ID NO: 62 - protein, 232 aa, synthetic construct
  source 1..232: note = Hinge region, CH2 domain, and CH3 domain without Knob mutation sites S354C and T366W
EPKSSDKTHTCPPCPAPELLGGPSVFLFPPKPKDTLMISRTPEVTCVVVDVSHEDPEVKFNWYVDGVEVHNAKTKPREEQYNSTYRVVSVLTVLHQDWLNGKEYKCKVSNKALPAPIEKTISKAKGQPREPQVYTLPPSRDELTKNQVSLTCLVKGFYPSDIAVEWESNGQPENNYKTTPPVLDSDGSFFLYSKLTVDKSRWQQGNVFSCSVMHEALHNHYTQKSLSLSPGK

SEQ ID NO: 63 - protein, 329 aa, synthetic construct
  source 1..329: note = Constant region sequence without hole mutation sites Y349C, T366S, L368A, and Y407V
ASTKGPSVFPLAPSSKSTSGGTAALGCLVKDYFPEPVTVSWNSGALTSGVHTFPAVLQSSGLYSLSSVVTVPSSSLGTQTYICNVNHKPSNTKVDKKVEPKSCDKTHTCPPCPAPELLGGPSVFLFPPKPKDTLMISRTPEVTCVVVDVSHEDPEVKFNWYVDGVEVHNAKTKPREEQYNSTYRVVSVLTVLHQDWLNGKEYKCKVSNKALPAPIEKTISKAKGQPREPQVYTLPPSRDELTKNQVSLTCLVKGFYPSDIAVEWESNGQPENNYKTTPPVLDSDGSFFLYSKLTVDKSRWQQGNVFSCSVMHEALHNHYTQKSLSLSPG

SEQ ID NO: 64 - protein, 444 aa, synthetic construct
  source 1..444: note = Amino acid sequence of the heavy chain of Hu5F9-G4
QVQLVQSGAEVKKPGASVKVSCKASGYTFTNYNMHWVRQAPGQRLEWMGTIYPGNDDTSYNQKFKDRVTITADTSASTAYMELSSLRSEDTAVYYCARGGYRAMDYWGQGTLVTVSSASTKGPSVFPLAPCSRSTSESTAALGCLVKDYFPEPVTVSWNSGALTSGVHTFPAVLQSSGLYSLSSVVTVPSSSLGTKTYTCNVDHKPSNTKVDKRVESKYGPPCPPCPAPEFLGGPSVFLFPPKPKDTLMISRTPEVTCVVVDVSQEDPEVQFNWYVDGVEVHNAKTKPREEQFNSTYRVVSVLTVLHQDWLNGKEYKCKVSNKGLPSSIEKTISKAKGQPREPQVYTLPPSQEEMTKNQVSLTCLVKGFYPSDIAVEWESNGQPENNYKTTPPVLDSDGSFFLYSRLTVDKSRWQEGNVFSCSVMHEALHNHYTQKSLSLSLGK

SEQ ID NO: 65 - protein, 219 aa, synthetic construct
  source 1..219: note = Amino acid sequence of the light chain of Hu5F9-G4
DIVMTQSPLSLPVTPGEPASISCRSSQSIVYSNGNTYLGWYLQKPGQSPQLLIYKVSNRFSGVPDRFSGSGSGTDFTLKISRVEAEDVGVYYCFQGSHVPYTFGQGTKLEIKRTVAAPSVFIFPPSDEQLKSGTASVVCLLNNFYPREAKVQWKVDNALQSGNSQESVTEQDSKDSTYSLSSTLTLSKADYEKHKVYACEVTHQGLSSPVTKSFNRGEC